European Patent Specification EP 3 371 217 B1, published June 11, 2025. Title: METHODS OF SCREENING FOR MULTISPECIFIC ANTIBODIES. Applicant: GENENTECH, INC. F. HOFFMANN-LA ROCHE AG. The sequence listing filed with the application follows.

SEQUENCE LISTING (88 sequences)

SEQ ID NO: 1 - protein, 992 aa, Homo sapiens
FSGDGRAIWSKNPNFTPVNESQLFLYDTFPKNFFWGIGTGALQVEGSWKKDGKGPSIWDHFIHTHLKNVSSTNGSSDSYIFLEKDLSALDFIGVSFYQFSISWPRLFPDGIVTVANAKGLQYYSTLLDALVLRNIEPIVTLYHWDLPLALQEKYGGWKNDTIIDIFNDYATYCFQMFGDRVKYWITIHNPYLVAWHGYGTGMHAPGEKGNLAAVYTVGHNLIKAHSKVWHNYNTHFRPHQKGWLSITLGSHWIEPNRSENTMDIFKCQQSMVSVLGWFANPIHGDGDYPEGMRKKLFSVLPIFSEAEKHEMRGTADFFAFSFGPNNFKPLNTMAKMGQNVSLNLREALNWIKLEYNNPRILIAENGWFTDSRVKTEDTTAIYMMKNFLSQVLQAIRLDEIRVFGYTAWSLLDGFEWQDAYTIRRGLFYVDFNSKQKERKPKSSAHYYKQIIRENGFSLKESTPDVQGQFPCDFSWGVTESVLKPESVASSPQFSDPHLYVWNATGNRLLHRVEGVRLKTRPAQCTDFVNIKKQLEMLARMKVTHYRFALDWASVLPTGNLSAVNRQALRYYRCVVSEGLKLGISAMVTLYYPTHAHLGLPEPLLHADGWLNPSTAEAFQAYAGLCFQELGDLVKLWITINEPNRLSDIYNRSGNDTYGAAHNLLVAHALAWRLYDRQFRPSQRGAVSLSLHADWAEPANPYADSHWRAAERFLQFEIAWFAEPLFKTGDYPAAMREYIASKHRRGLSSSALPRLTEAERRLLKGTVDFCALNHFTTRFVMHEQLAGSRYDSDRDIQFLQDITRLSSPTRLAVIPWGVRKLLRWVRRNYGDMDIYITASGIDDQALEDDRLRKYYLGKYLQEVLKAYLIDKVRIKGYYAFKLAEEKSKPRFGFFTSDFKAKSSIQFYNKVISSRGFPFENSSSRCSQTQENTECTVCLFLVQKKPLIFLGCCFFSTLVLLLSIAIFQRQKRRKFWKAKNLQHIPLKKGKRVVS

SEQ ID NO: 2 - protein, 455 aa, Homo sapiens
FPCDFSWGVTESVLKPESVASSPQFSDPHLYVWNATGNRLLHRVEGVRLKTRPAQCTDFVNIKKQLEMLARMKVTHYRFALDWASVLPTGNLSAVNRQALRYYRCVVSEGLKLGISAMVTLYYPTHAHLGLPEPLLHADGWLNPSTAEAFQAYAGLCFQELGDLVKLWITINEPNRLSDIYNRSGNDTYGAAHNLLVAHALAWRLYDRQFRPSQRGAVSLSLHADWAEPANPYADSHWRAAERFLQFEIAWFAEPLFKTGDYPAAMREYIASKHRRGLSSSALPRLTEAERRLLKGTVDFCALNHFTTRFVMHEQLAGSRYDSDRDIQFLQDITRLSSPTRLAVIPWGVRKLLRWVRRNYGDMDIYITASGIDDQALEDDRLRKYYLGKYLQEVLKAYLIDKVRIKGYYAFKLAEEKSKPRFGFFTSDFKAKSSIQFYNKVISSRGFPFENSSSR

SEQ ID NO: 3 - protein, 5 aa, Artificial Sequence
  source: /note="Description of Artificial Sequence: Synthetic peptide"
NYGMN

SEQ ID NO: 4 - protein, 6 aa, Artificial Sequence
  source: /note="Description of Artificial Sequence: Synthetic peptide"
SGYYWT

SEQ ID NO: 5 - protein, 5 aa, Artificial Sequence
  source: /note="Description of Artificial Sequence: Synthetic peptide"
NYDIN

SEQ ID NO: 6 - protein, 6 aa, Artificial Sequence
  source: /note="Description of Artificial Sequence: Synthetic peptide"
SGYYWN

SEQ ID NO: 7 - protein, 5 aa, Artificial Sequence
  source: /note="Description of Artificial Sequence: Synthetic peptide"
DYYIN

SEQ ID NO: 8 - protein, 17 aa, Artificial Sequence
  source: /note="Description of Artificial Sequence: Synthetic peptide"
WIDTDTGEATYTDDFKG

SEQ ID NO: 9 - protein, 16 aa, Artificial Sequence
  source: /note="Description of Artificial Sequence: Synthetic peptide"
YIKYDGGNYYNPSLRN

SEQ ID NO: 10 - protein, 17 aa, Artificial Sequence
  source: /note="Description of Artificial Sequence: Synthetic peptide"
WIYPRDGSAKYNAKFKG

SEQ ID NO: 11 - protein, 16 aa, Artificial Sequence
  source: /note="Description of Artificial Sequence: Synthetic peptide"
YIRYDGNSNYNPFLKN

SEQ ID NO: 12 - protein, 17 aa, Artificial Sequence
  source: /note="Description of Artificial Sequence: Synthetic peptide"
DINPNNGDTTYNQKFKA

SEQ ID NO: 13 - protein, 10 aa, Artificial Sequence
  source: /note="Description of Artificial Sequence: Synthetic peptide"
EEYGLFGFPY

SEQ ID NO: 14 - protein, 13 aa, Artificial Sequence
  source: /note="Description of Artificial Sequence: Synthetic peptide"
GDYYASPYGAMDS

SEQ ID NO: 15 - protein, 14 aa, Artificial Sequence
  source: /note="Description of Artificial Sequence: Synthetic peptide"
RPLYYGSTHWYFDV

SEQ ID NO: 16 - protein, 13 aa, Artificial Sequence
  source: /note="Description of Artificial Sequence: Synthetic peptide"
KGAYYSSFDALDY

SEQ ID NO: 17 - protein, 9 aa, Artificial Sequence
  source: /note="Description of Artificial Sequence: Synthetic peptide"
RFYSSPFDS

SEQ ID NO: 18 - protein, 11 aa, Artificial Sequence
  source: /note="Description of Artificial Sequence: Synthetic peptide"
KASEDIYNRLA

SEQ ID NO: 19 - protein, 11 aa, Artificial Sequence
  source: /note="Description of Artificial Sequence: Synthetic peptide"
HASQDIDVWLS

SEQ ID NO: 20 - protein, 15 aa, Artificial Sequence
  source: /note="Description of Artificial Sequence: Synthetic peptide"
KASQSVDYDGDSYMN

SEQ ID NO: 21 - protein, 11 aa, Artificial Sequence
  source: /note="Description of Artificial Sequence: Synthetic peptide"
KASQDIRSYLS

SEQ ID NO: 22 - protein, 17 aa, Artificial Sequence
  source: /note="Description of Artificial Sequence: Synthetic peptide"
KSGQSLLYSRNQKNYLA

SEQ ID NO: 23 - protein, 7 aa, Artificial Sequence
  source: /note="Description of Artificial Sequence: Synthetic peptide"
AATSLET

SEQ ID NO: 24 - protein, 7 aa, Artificial Sequence
  source: /note="Description of Artificial Sequence: Synthetic peptide"
KSSILHT

SEQ ID NO: 25 - protein, 7 aa, Artificial Sequence
  source: /note="Description of Artificial Sequence: Synthetic peptide"
AASNLKS

SEQ ID NO: 26 - protein, 7 aa, Artificial Sequence
  source: /note="Description of Artificial Sequence: Synthetic peptide"
RANRLVD

SEQ ID NO: 27 - protein, 7 aa, Artificial Sequence
  source: /note="Description of Artificial Sequence: Synthetic peptide"
WASTRES

SEQ ID NO: 28 - protein, 9 aa, Artificial Sequence
  source: /note="Description of Artificial Sequence: Synthetic peptide"
QQYWSNPLT

SEQ ID NO: 29 - protein, 9 aa, Artificial Sequence
  source: /note="Description of Artificial Sequence: Synthetic peptide"
QQGLSYPFT

SEQ ID NO: 30 - protein, 9 aa, Artificial Sequence
  source: /note="Description of Artificial Sequence: Synthetic peptide"
QQSNEDPRT

SEQ ID NO: 31 - protein, 9 aa, Artificial Sequence
  source: /note="Description of Artificial Sequence: Synthetic peptide"
LQYDEFPLT

SEQ ID NO: 32 - protein, 9 aa, Artificial Sequence
  source: /note="Description of Artificial Sequence: Synthetic peptide"
QQYYSYPYT

SEQ ID NO: 33 - protein, 107 aa, Artificial Sequence
  source: /note="Description of Artificial Sequence: Synthetic polypeptide"
DIQMTQSSSSFSVSLGDRVTITCKASEDIYNRLAWYQQKPGSAPRLLISAATSLETGVPSRFSGSGSGKDYTLSITSLQTEDVATYYCQQYWSNPLTFGAGTKLELK

SEQ ID NO: 34 - protein, 119 aa, Artificial Sequence
  source: /note="Description of Artificial Sequence: Synthetic polypeptide"
QIQLVQSGPELKKPGETAKISCKASGYAFSNYGMNWVKQAPGKDLKWMGWIDTDTGEATYTDDFKGRFVFSLETSASTAYLQINNLKNEDMATYFCAREEYGLFGFPYWGHGTLVTVSA

SEQ ID NO: 35 - protein, 107 aa, Artificial Sequence
  source: /note="Description of Artificial Sequence: Synthetic polypeptide"
DIVMTQSPSSLSASLGDTITITCHASQDIDVWLSWYQQKPGNVPQLLISKSSILHTGVPSRFSGGGSGTGFTLTISSLQPEDIATYYCQQGLSYPFTFGSGTKLKIK

SEQ ID NO: 36 - protein, 122 aa, Artificial Sequence
  source: /note="Description of Artificial Sequence: Synthetic polypeptide"
EVQLQQSGPGLVKPSQSLSLTCSVTGYSITSGYYWTWIRQFPGNKLEWMGYIKYDGGNYYNPSLRNRISITRDTSKNHFFLKFYSVTAEDTATYFCARGDYYASPYGAMDSWGQGTSVTVSS

SEQ ID NO: 37 - protein, 111 aa, Artificial Sequence
  source: /note="Description of Artificial Sequence: Synthetic polypeptide"
DIVLTQSPASLAVSLGQRATISCKASQSVDYDGDSYMNWYQQKPGQPPKLLIYAASNLKSGIPARFSGSGSGTDFTLNIHPVEEEDAATYYCQQSNEDPRTFGGGTRLEIK

SEQ ID NO: 38 - protein, 123 aa, Artificial Sequence
  source: /note="Description of Artificial Sequence: Synthetic polypeptide"
QVQLQQSGPELVKPGASVKLSCKASGYTFTNYDINWVRQRPGQGLEWIGWIYPRDGSAKYNAKFKGKATLTVDTSSSTAYMELHSLTSEDSAVYFCARRPLYYGSTHWYFDVWGTGTTVTVSS

SEQ ID NO: 39 - protein, 107 aa, Artificial Sequence
  source: /note="Description of Artificial Sequence: Synthetic polypeptide"
DIVMTQSPSSMYASLGERVTISCKASQDIRSYLSWFQQKPGKSPKTLIYRANRLVDGVPSRFSGSGSGQDYSLTITSLEFGDVGLYYCLQYDEFPLTFGAGTKLKIE

SEQ ID NO: 40 - protein, 122 aa, Artificial Sequence
  source: /note="Description of Artificial Sequence: Synthetic polypeptide"
EVQLQESGPGLVKPSQSLSLTCSVTGYSITSGYYWNWIRQFPGNKLEWMGYIRYDGNSNYNPFLKNRVSITRDTSKNQFFLKLNSVTTEDTATYYCTRKGAYYSSFDALDYWGQGTSVTVSS

SEQ ID NO: 41 - protein, 113 aa, Artificial Sequence
  source: /note="Description of Artificial Sequence: Synthetic polypeptide"
DIVMTQSPSSLAVSVGEKVTLSCKSGQSLLYSRNQKNYLAWYQQKPGQSPKLLISWASTRESGVPDRFTGSGSGTDFTLTISSVKTEDLAVYHCQQYYSYPYTFGGGTRLEIK

SEQ ID NO: 42 - protein, 118 aa, Artificial Sequence
  source: /note="Description of Artificial Sequence: Synthetic polypeptide"
EVQLQQSGPELVQPGTSVKISCEASGYTFTDYYINWVKQSRGKSLEWIGDINPNNGDTTYNQKFKAKATLTVDRSSNTAYMELRSLTSEDSVVYYCARRFYSSPFDSWGQGTTLTVSS

SEQ ID NO: 43 - protein, 90 aa, Homo sapiens
IQFYNKVISSRGFPFENSSSRCSQTQENTECTVCLFLVQKKPLIFLGCCFFSTLVLLLSIAIFQRQKRRKFWKAKNLQHIPLKKGKRVVS

SEQ ID NO: 44 - protein, 94 aa, Homo sapiens
ADSHWRAAERFLQFEIAWFAEPLFKTGDYPAAMREYIASKHRRGLSSSALPRLTEAERRLLKGTVDFCALNHFTTRFVMHEQLAGSRYDSDRDI

SEQ ID NO: 45 - protein, 567 aa, Homo sapiens
FSGDGRAIWSKNPNFTPVNESQLFLYDTFPKNFFWGIGTGALQVEGSWKKDGKGPSIWDHFIHTHLKNVSSTNGSSDSYIFLEKDLSALDFIGVSFYQFSISWPRLFPDGIVTVANAKGLQYYSTLLDALVLRNIEPIVTLYHWDLPLALQEKYGGWKNDTIIDIFNDYATYCFQMFGDRVKYWITIHNPYLVAWHGYGTGMHAPGEKGNLAAVYTVGHNLIKAHSKVWHNYNTHFRPHQKGWLSITLGSHWIEPNRSENTMDIFKCQQSMVSVLGWFANPIHGDGDYPEGMRKKLFSVLPIFSEAEKHEMRGTADFFAFSFGPNNFKPLNTMAKMGQNVSLNLREALNWIKLEYNNPRILIAENGWFTDSRVKTEDTTAIYMMKNFLSQVLQAIRLDEIRVFGYTAWSLLDGFEWQDAYTIRRGLFYVDFNSKQKERKPKSSAHYYKQIIRENGFSLKESTPDVQGQFPCDFSWGVTESVLKPESVASSPQFSDPHLYVWNATGNRLLHRVEGVRLKTRPAQCTDFVNIKKQLEMLARMKVTHYRFALDWASVLPTGNLSAVNRQA

SEQ ID NO: 46 - protein, 106 aa, Homo sapiens
KTVALGSNVEFMCKVYSDPQPHIQWLKHIEVNGSKIGPDNLPYVQILKTAGVNTTDKEMEVLHLRNVSFEDAGEYTCLAGNSIGLSHHSAWLTVLEALEERPAVMT

SEQ ID NO: 47 - protein, 992 aa, Homo sapiens; identical to SEQ ID NO: 1

SEQ ID NO: 48 - protein, 991 aa, Rattus sp.
FSGDGKAIWDKKQYVSPVNPGQLFLYDTFPKNFSWGVGTGAFQVEGSWKADGRGPSIWDRYVDSHLRGVNSTDRSTDSYVFLEKDLLALDFLGVSFYQFSISWPRLFPNGTVAAVNAKGLQYYRALLDSLVLRNIEPIVTLYHWDLPLTLQEEYGGWKNATMIDLFNDYATYCFQTFGDRVKYWITIHNPYLVAWHGFGTGMHAPGEKGNLTAVYTVGHNLIKAHSKVWHNYDKNFRPHQKGWLSITLGSHWIEPNRTENMEDVINCQHSMSSVLGWFANPIHGDGDYPEFMKTSSVIPEFSEAEKEEVRGTADFFAFSFGPNNFRPSNTVVKMGQNVSLNLRQVLNWIKLEYDNPRILISENGWFTDSYIKTEDTTAIYMMKNFLNQVLQAIKFDEIQVFGYTAWTLLDGFEWQDAYTTRRGLFYVDFNSEQKERKPKSSAHYYKQIIQDNGFPLQESTPDMKGQFPCDFSWGVTESVLKPEFTVSSPQFTDPHLYVWNVTGNRLLYRVEGVRLKTRPSQCTDYVSIKKRVEMLAKMKVTHYQFALDWTSILPTGNLSKINRQVLRYYRCVVSEGLKLGISPMVTLYHPTHSHLGLPMPLLSSGGWLNTNTAKAFQDYAGLCFKELGDLVKLWITINEPNRLSDMYNRTSNDTYRAAHNLMIAHAQVWHLYDRQYRPVQHGAVSLSLHSDWAEPANPYVESHWKAAERFLQFEIAWFADPLFKTGDYPLAMKEYIASKKQRGLSSSVLPRFTLKESRLVKGTIDFYALNHFTTRFVIHKQLNTNCSVADRDVQFLQDITRLSSPSRLAVTPWGMRKLLGWIRRNYRDMDIYVTANGIDDLALEDDQIRKYYLEKYVQEALKAYLIDKVKIKGYYAFKLTEEKSKPRFGFFTSDFKAKSSVQFYSKLISSSGFSSENRSPACGQPPEDTECAICSFLTQKKPLIFFGCCFISTLAALLSITIFHHRKRRKFQKARNLQNIPLKKGHSRVFS

SEQ ID NO: 49 - protein, 993 aa, Artificial Sequence
  source: /note="Description of Artificial Sequence: Synthetic polypeptide"
FSGDGRAIWSKNPNFTPVNESQLFLYDTFPKNFFWGIGTGALQVEGSWKKDGKGPSIWDHFIHTHLKNVSSTNGSSDSYIFLEKDLSALDFIGVSFYQFSISWPRLFPDGIVTVANAKGLQYYSTLLDALVLRNIEPIVTLYHWDLPLALQEKYGGWKNDTIIDIFNDYATYCFQMFGDRVKYWITIHNPYLVAWHGYGTGMHAPGEKGNLAAVYTVGHNLIKAHSKVWHNYNTHFRPHQKGWLSITLGSHWIEPNRSENTMDIFKCQQSMVSVLGWFANPIHGDGDYPEGMRKKLFSVLPIFSEAEKHEMRGTADFFAFSFGPNNFKPLNTMAKMGQNVSLNLREALNWIKLEYNNPRILIAENGWFTDSRVKTEDTTAIYMMKNFLSQVLQAIRLDEIRVFGYTAWSLLDGFEWQDAYTIRRGLFYVDFNSKQKERKPKSSAHYYKQIIRENGFSLKESTPDVQGQFPCDFSWGVTESVLKPESVASSPQFSDPHLYVWNATGNRLLHRVEGVRLKTRPAQCTDFVNIKKQLEMLARMKVTHYRFALDWASVLPTGNLSAVNRQALRYYRCVVSEGLKLGISAMVTLYHPTHSHLGLPMPLLSSGGWLNTNTAKAFQDYAGLCFKELGDLVKLWITINEPNRLSDMYNRTSNDTYRAAHNLMIAHAQVWHLYDRQYRPVQHGAVSLSLHSDWAEPANPYVESHWKAAERFLQFEIAWFADPLFKTGDYPLAMKEYIASKKQRGLSSSVLPRFTLKESRLVKGTIDFYALNHFTTRFVIHKQLNTNCSVADRDVQFLQDITRLSSPSRLAVTPWGMRKLLGWIRRNYRDMDIYVTANGIDDLALEDDQIRKYYLEKYVQEALKAYLIDKVKIKGYYAFKLTEEKSKPRFGFFTSDFKAKSSVQFYSKLISSSGFSSENRSPACGQPPEDTECAICSFLTQKKPLIFFGCCFISTLAALLSITIFHHRKRRKFQKARNLQNIPLKKGHSRVFS

SEQ ID NO: 50 - protein, 993 aa, Artificial Sequence
  source: /note="Description of Artificial Sequence: Synthetic polypeptide"
FSGDGRAIWSKNPNFTPVNESQLFLYDTFPKNFFWGIGTGALQVEGSWKKDGKGPSIWDHFIHTHLKNVSSTNGSSDSYIFLEKDLSALDFIGVSFYQFSISWPRLFPDGIVTVANAKGLQYYSTLLDALVLRNIEPIVTLYHWDLPLALQEKYGGWKNDTIIDIFNDYATYCFQMFGDRVKYWITIHNPYLVAWHGYGTGMHAPGEKGNLAAVYTVGHNLIKAHSKVWHNYNTHFRPHQKGWLSITLGSHWIEPNRSENTMDIFKCQQSMVSVLGWFANPIHGDGDYPEGMRKKLFSVLPIFSEAEKHEMRGTADFFAFSFGPNNFKPLNTMAKMGQNVSLNLREALNWIKLEYNNPRILIAENGWFTDSRVKTEDTTAIYMMKNFLSQVLQAIRLDEIRVFGYTAWSLLDGFEWQDAYTIRRGLFYVDFNSKQKERKPKSSAHYYKQIIRENGFSLKESTPDVQGQFPCDFSWGVTESVLKPESVASSPQFSDPHLYVWNATGNRLLHRVEGVRLKTRPAQCTDFVNIKKQLEMLARMKVTHYRFALDWASVLPTGNLSAVNRQALRYYRCVVSEGLKLGISAMVTLYYPTHAHLGLPEPLLHADGWLNPSTAEAFQAYAGLCFQELGDLVKLWITINEPNRLSDIYNRSGNDTYGAAHNLLVAHALAWRLYDRQFRPSQRGAVSLSLHADWAEPANPYVESHWKAAERFLQFEIAWFADPLFKTGDYPLAMKEYIASKKQRGLSSSVLPRFTLKESRLVKGTIDFYALNHFTTRFVIHKQLNTNCSVADRDVQFLQDITRLSSPSRLAVTPWGMRKLLGWIRRNYRDMDIYVTANGIDDLALEDDQIRKYYLEKYVQEALKAYLIDKVKIKGYYAFKLTEEKSKPRFGFFTSDFKAKSSVQFYSKLISSSGFSSENRSPACGQPPEDTECAICSFLTQKKPLIFFGCCFISTLAALLSITIFHHRKRRKFQKARNLQNIPLKKGHSRVFS

SEQ ID NO: 51 - protein, 993 aa, Artificial Sequence
  source: /note="Description of Artificial Sequence: Synthetic polypeptide"
FSGDGRAIWSKNPNFTPVNESQLFLYDTFPKNFFWGIGTGALQVEGSWKKDGKGPSIWDHFIHTHLKNVSSTNGSSDSYIFLEKDLSALDFIGVSFYQFSISWPRLFPDGIVTVANAKGLQYYSTLLDALVLRNIEPIVTLYHWDLPLALQEKYGGWKNDTIIDIFNDYATYCFQMFGDRVKYWITIHNPYLVAWHGYGTGMHAPGEKGNLAAVYTVGHNLIKAHSKVWHNYNTHFRPHQKGWLSITLGSHWIEPNRSENTMDIFKCQQSMVSVLGWFANPIHGDGDYPEGMRKKLFSVLPIFSEAEKHEMRGTADFFAFSFGPNNFKPLNTMAKMGQNVSLNLREALNWIKLEYNNPRILIAENGWFTDSRVKTEDTTAIYMMKNFLSQVLQAIRLDEIRVFGYTAWSLLDGFEWQDAYTIRRGLFYVDFNSKQKERKPKSSAHYYKQIIRENGFSLKESTPDVQGQFPCDFSWGVTESVLKPESVASSPQFSDPHLYVWNATGNRLLHRVEGVRLKTRPAQCTDFVNIKKQLEMLARMKVTHYRFALDWASVLPTGNLSAVNRQALRYYRCVVSEGLKLGISAMVTLYYPTHAHLGLPEPLLHADGWLNPSTAEAFQAYAGLCFQELGDLVKLWITINEPNRLSDIYNRSGNDTYGAAHNLLVAHALAWRLYDRQFRPSQRGAVSLSLHADWAEPANPYADSHWRAAERFLQFEIAWFAEPLFKTGDYPAAMREYIASKHRRGLSSSALPRLTEAERRLLKGTVDFCALNHFTTRFVMHEQLAGSRYDSDRDIQFLQDITRLSSPSRLAVTPWGMRKLLGWIRRNYRDMDIYVTANGIDDLALEDDQIRKYYLEKYVQEALKAYLIDKVKIKGYYAFKLTEEKSKPRFGFFTSDFKAKSSVQFYSKLISSSGFSSENRSPACGQPPEDTECAICSFLTQKKPLIFFGCCFISTLAALLSITIFHHRKRRKFQKARNLQNIPLKKGHSRVFS

SEQ ID NO: 52 - protein, 990 aa, Artificial Sequence
  source: /note="Description of Artificial Sequence: Synthetic polypeptide"
FSGDGKAIWDKKQYVSPVNPGQLFLYDTFPKNFSWGVGTGAFQVEGSWKADGRGPSIWDRYVDSHLRGVNSTDRSTDSYVFLEKDLLALDFLGVSFYQFSISWPRLFPNGTVAAVNAKGLQYYRALLDSLVLRNIEPIVTLYHWDLPLTLQEEYGGWKNATMIDLFNDYATYCFQTFGDRVKYWITIHNPYLVAWHGFGTGMHAPGEKGNLTAVYTVGHNLIKAHSKVWHNYDKNFRPHQKGWLSITLGSHWIEPNRTENMEDVINCQHSMSSVLGWFANPIHGDGDYPEFMKTSSVIPEFSEAEKEEVRGTADFFAFSFGPNNFRPSNTVVKMGQNVSLNLRQVLNWIKLEYDNPRILISENGWFTDSYIKTEDTTAIYMMKNFLNQVLQAIKFDEIQVFGYTAWTLLDGFEWQDAYTTRRGLFYVDFNSEQKERKPKSSAHYYKQIIQDNGFPLQESTPDMKGQFPCDFSWGVTESVLKPEFTVSSPQFTDPHLYVWNVTGNRLLYRVEGVRLKTRPSQCTDYVSIKKRVEMLAKMKVTHYQFALDWTSILPTGNLSKINRQVLRYYRCVVSEGLKLGISPMVTLYHPTHSHLGLPMPLLSSGGWLNTNTAKAFQDYAGLCFKELGDLVKLWITINEPNRLSDMYNRTSNDTYRAAHNLMIAHAQVWHLYDRQYRPVQHGAVSLSLHSDWAEPANPYVESHWKAAERFLQFEIAWFADPLFKTGDYPLAMKEYIASKKQRGLSSSVLPRFTLKESRLVKGTIDFYALNHFTTRFVIHKQLNTNCSVADRDVQFLQDITRLSSPTRLAVIPWGVRKLLRWVRRNYGDMDIYITASGIDDQALEDDRLRKYYLGKYLQEVLKAYLIDKVRIKGYYAFKLAEEKSKPRFGFFTSDFKAKSSIQFYNKVISSRGFPFENSSSRCSQTQENTECTVCLFLVQKKPLIFLGCCFFSTLVLLLSIAIFQRQKRRKFWKAKNLQHIPLKKGKRVVS

SEQ ID NO: 53 - protein, 990 aa, Artificial Sequence
  source: /note="Description of Artificial Sequence: Synthetic polypeptide"
FSGDGKAIWDKKQYVSPVNPGQLFLYDTFPKNFSWGVGTGAFQVEGSWKADGRGPSIWDRYVDSHLRGVNSTDRSTDSYVFLEKDLLALDFLGVSFYQFSISWPRLFPNGTVAAVNAKGLQYYRALLDSLVLRNIEPIVTLYHWDLPLTLQEEYGGWKNATMIDLFNDYATYCFQTFGDRVKYWITIHNPYLVAWHGFGTGMHAPGEKGNLTAVYTVGHNLIKAHSKVWHNYDKNFRPHQKGWLSITLGSHWIEPNRTENMEDVINCQHSMSSVLGWFANPIHGDGDYPEFMKTSSVIPEFSEAEKEEVRGTADFFAFSFGPNNFRPSNTVVKMGQNVSLNLRQVLNWIKLEYDNPRILISENGWFTDSYIKTEDTTAIYMMKNFLNQVLQAIKFDEIQVFGYTAWTLLDGFEWQDAYTTRRGLFYVDFNSEQKERKPKSSAHYYKQIIQDNGFPLQESTPDMKGQFPCDFSWGVTESVLKPEFTVSSPQFTDPHLYVWNVTGNRLLYRVEGVRLKTRPSQCTDYVSIKKRVEMLAKMKVTHYQFALDWTSILPTGNLSKINRQVLRYYRCVVSEGLKLGISPMVTLYHPTHSHLGLPMPLLSSGGWLNTNTAKAFQDYAGLCFKELGDLVKLWITINEPNRLSDMYNRTSNDTYRAAHNLMIAHAQVWHLYDRQYRPVQHGAVSLSLHSDWAEPANPYVESHWKAAERFLQFEIAWFADPLFKTGDYPLAMKEYIASKKQRGLSSSVLPRFTLKESRLVKGTIDFYALNHFTTRFVIHKQLNTNCSVADRDVQFLQDITRLSSPSRLAVTPWGMRKLLGWIRRNYRDMDIYVTANGIDDQALEDDRLRKYYLGKYLQEVLKAYLIDKVRIKGYYAFKLAEEKSKPRFGFFTSDFKAKSSIQFYNKVISSRGFPFENSSSRCSQTQENTECTVCLFLVQKKPLIFLGCCFFSTLVLLLSIAIFQRQKRRKFWKAKNLQHIPLKKGKRVVS

SEQ ID NO: 54 - protein, 990 aa, Artificial Sequence
  source: /note="Description of Artificial Sequence: Synthetic polypeptide"
FSGDGKAIWDKKQYVSPVNPGQLFLYDTFPKNFSWGVGTGAFQVEGSWKADGRGPSIWDRYVDSHLRGVNSTDRSTDSYVFLEKDLLALDFLGVSFYQFSISWPRLFPNGTVAAVNAKGLQYYRALLDSLVLRNIEPIVTLYHWDLPLTLQEEYGGWKNATMIDLFNDYATYCFQTFGDRVKYWITIHNPYLVAWHGFGTGMHAPGEKGNLTAVYTVGHNLIKAHSKVWHNYDKNFRPHQKGWLSITLGSHWIEPNRTENMEDVINCQHSMSSVLGWFANPIHGDGDYPEFMKTSSVIPEFSEAEKEEVRGTADFFAFSFGPNNFRPSNTVVKMGQNVSLNLRQVLNWIKLEYDNPRILISENGWFTDSYIKTEDTTAIYMMKNFLNQVLQAIKFDEIQVFGYTAWTLLDGFEWQDAYTTRRGLFYVDFNSEQKERKPKSSAHYYKQIIQDNGFPLQESTPDMKGQFPCDFSWGVTESVLKPEFTVSSPQFTDPHLYVWNVTGNRLLYRVEGVRLKTRPSQCTDYVSIKKRVEMLAKMKVTHYQFALDWTSILPTGNLSKINRQVLRYYRCVVSEGLKLGISPMVTLYHPTHSHLGLPMPLLSSGGWLNTNTAKAFQDYAGLCFKELGDLVKLWITINEPNRLSDMYNRTSNDTYRAAHNLMIAHAQVWHLYDRQYRPVQHGAVSLSLHSDWAEPANPYVESHWKAAERFLQFEIAWFADPLFKTGDYPLAMKEYIASKKQRGLSSSVLPRFTLKESRLVKGTIDFYALNHFTTRFVIHKQLNTNCSVADRDVQFLQDITRLSSPSRLAVTPWGMRKLLGWIRRNYRDMDIYVTANGIDDLALEDDQIRKYYLEKYVQEALKAYLIDKVKIKGYYAFKLTEEKSKPRFGFFTSDFKAKSSIQFYNKVISSRGFPFENSSSRCSQTQENTECTVCLFLVQKKPLIFLGCCFFSTLVLLLSIAIFQRQKRRKFWKAKNLQHIPLKKGKRVVS

SEQ ID NO: 55 - protein, 991 aa, Artificial Sequence
  source: /note="Description of Artificial Sequence: Synthetic polypeptide"
FSGDGKAIWDKKQYVSPVNPGQLFLYDTFPKNFSWGVGTGAFQVEGSWKADGRGPSIWDRYVDSHLRGVNSTDRSTDSYVFLEKDLLALDFLGVSFYQFSISWPRLFPNGTVAAVNAKGLQYYRALLDSLVLRNIEPIVTLYHWDLPLTLQEEYGGWKNATMIDLFNDYATYCFQTFGDRVKYWITIHNPYLVAWHGFGTGMHAPGEKGNLTAVYTVGHNLIKAHSKVWHNYDKNFRPHQKGWLSITLGSHWIEPNRTENMEDVINCQHSMSSVLGWFANPIHGDGDYPEFMKTSSVIPEFSEAEKEEVRGTADFFAFSFGPNNFRPSNTVVKMGQNVSLNLRQVLNWIKLEYDNPRILISENGWFTDSYIKTEDTTAIYMMKNFLNQVLQAIKFDEIQVFGYTAWTLLDGFEWQDAYTTRRGLFYVDFNSEQKERKPKSSAHYYKQIIQDNGFPLQESTPDMKGQFPCDFSWGVTESVLKPEFTVSSPQFTDPHLYVWNVTGNRLLYRVEGVRLKTRPSQCTDYVSIKKRVEMLAKMKVTHYQFALDWTSILPTGNLSKINRQVLRYYRCVVSEGLKLGISPMVTLYHPTHSHLGLPMPLLSSGGWLNTNTAKAFQDYAGLCFKELGDLVKLWITINEPNRLSDMYNRTSNDTYRAAHNLMIAHAQVWHLYDRQYRPVQHGAVSLSLHSDWAEPANPYVESHWKAAERFLQFEIAWFADPLFKTGDYPLAMKEYIASKKQRGLSSSVLPRFTLKESRLVKGTIDFYALNHFTTRFVIHKQLNTNCSVADRDVQFLQDITRLSSPTRLAVIPWGVRKLLRWVRRNYGDMDIYITASGIDDQALEDDRLRKYYLGKYLQEVLKAYLIDKVRIKGYYAFKLAEEKSKPRFGFFTSDFKAKSSVQFYSKLISSSGFSSENRSPACGQPPEDTECAICSFLTQKKPLIFFGCCFISTLAALLSITIFHHRKRRKFQKARNLQNIPLKKGHSRVFS

SEQ ID NO: 56 - protein, 991 aa, Artificial Sequence
  source: /note="Description of Artificial Sequence: Synthetic polypeptide"
FSGDGKAIWDKKQYVSPVNPGQLFLYDTFPKNFSWGVGTGAFQVEGSWKADGRGPSIWDRYVDSHLRGVNSTDRSTDSYVFLEKDLLALDFLGVSFYQFSISWPRLFPNGTVAAVNAKGLQYYRALLDSLVLRNIEPIVTLYHWDLPLTLQEEYGGWKNATMIDLFNDYATYCFQTFGDRVKYWITIHNPYLVAWHGFGTGMHAPGEKGNLTAVYTVGHNLIKAHSKVWHNYDKNFRPHQKGWLSITLGSHWIEPNRTENMEDVINCQHSMSSVLGWFANPIHGDGDYPEFMKTSSVIPEFSEAEKEEVRGTADFFAFSFGPNNFRPSNTVVKMGQNVSLNLRQVLNWIKLEYDNPRILISENGWFTDSYIKTEDTTAIYMMKNFLNQVLQAIKFDEIQVFGYTAWTLLDGFEWQDAYTTRRGLFYVDFNSEQKERKPKSSAHYYKQIIQDNGFPLQESTPDMKGQFPCDFSWGVTESVLKPEFTVSSPQFTDPHLYVWNVTGNRLLYRVEGVRLKTRPSQCTDYVSIKKRVEMLAKMKVTHYQFALDWTSILPTGNLSKINRQVLRYYRCVVSEGLKLGISPMVTLYHPTHSHLGLPMPLLSSGGWLNTNTAKAFQDYAGLCFKELGDLVKLWITINEPNRLSDMYNRTSNDTYRAAHNLMIAHAQVWHLYDRQYRPVQHGAVSLSLHSDWAEPANPYVESHWKAAERFLQFEIAWFADPLFKTGDYPLAMKEYIASKKQRGLSSSVLPRFTLKESRLVKGTIDFYALNHFTTRFVIHKQLNTNCSVADRDVQFLQDITRLSSPTRLAVIPWGVRKLLRWVRRNYGDMDIYITASGIDDLALEDDQIRKYYLEKYVQEALKAYLIDKVKIKGYYAFKLTEEKSKPRFGFFTSDFKAKSSVQFYSKLISSSGFSSENRSPACGQPPEDTECAICSFLTQKKPLIFFGCCFISTLAALLSITIFHHRKRRKFQKARNLQNIPLKKGHSRVFS

SEQ ID NO: 57 - protein, 799 aa, Homo sapiens
RPSPTLPEQAQPWGAPVEVESFLVHPGDLLQLRCRLRDDVQSINWLRDGVQLAESNRTRITGEEVEVQDSVPADSGLYACVTSSPSGSDTTYFSVNVSDALPSSEDDDDDDDSSSEEKETDNTKPNPVAPYWTSPEKMEKKLHAVPAAKTVKFKCPSSGTPNPTLRWLKNGKEFKPDHRIGGYKVRYATWSIIMDSVVPSDKGNYTCIVENEYGSINHTYQLDVVERSPHRPILQAGLPANKTVALGSNVEFMCKVYSDPQPHIQWLKHIEVNGSKIGPDNLPYVQILKTAGVNTTDKEMEVLHLRNVSFEDAGEYTCLAGNSIGLSHHSAWLTVLEALEERPAVMTSPLYLEIIIYCTGAFLISCMVGSVIVYKMKSGTKKSDFHSQMAVHKLAKSIPLRRQVTVSADSSASMNSGVLLVRPSRLSSSGTPMLAGVSEYELPEDPRWELPRDRLVLGKPLGEGCFGQVVLAEAIGLDKDKPNRVTKVAVKMLKSDATEKDLSDLISEMEMMKMIGKHKNIINLLGACTQDGPLYVIVEYASKGNLREYLQARRPPGLEYCYNPSHNPEEQLSSKDLVSCAYQVARGMEYLASKKCIHRDLAARNVLVTEDNVMKIADFGLARDIHHIDYYKKTTNGRLPVKWMAPEALFDRIYTHQSDVWSFGVLLWEIFTLGGSPYPGVPVEELFKLLKEGHRMDKPSNCTNELYMMMRDCWHAVPSQRPTFKQLVEDLDRIVALTSNQEYLDLSMPLDQYSPSFPDTRSSTCSSGEDSVFSHEPLPEEPCLPRHPAQLANGGLKRR

SEQ ID NO: 58 - protein, 800 aa, Homo sapiens
RPSFSLVEDTTLEPEEPPTKYQISQPEVYVAAPGESLEVRCLLKDAAVISWTKDGVHLGPNNRTVLIGEYLQIKGATPRDSGLYACTASRTVDSETWYFMVNVTDAISSGDDEDDTDGAEDFVSENSNNKRAPYWTNTEKMEKRLHAVPAANTVKFRCPAGGNPMPTMRWLKNGKEFKQEHRIGGYKVRNQHWSLIMESVVPSDKGNYTCVVENEYGSINHTYHLDVVERSPHRPILQAGLPANASTVVGGDVEFVCKVYSDAQPHIQWIKHVEKNGSKYGPDGLPYLKVLKAAGVNTTDKEIEVLYIRNVTFEDAGEYTCLAGNSIGISFHSAWLTVLPAPGREKEITASPDYLEIAIYCIGVFLIACMVVTVILCRMKNTTKKPDFSSQPAVHKLTKRIPLRRQVTVSAESSSSMNSNTPLVRITTRLSSTADTPMLAGVSEYELPEDPKWEFPRDKLTLGKPLGEGCFGQVVMAEAVGIDKDKPKEAVTVAVKMLKDDATEKDLSDLVSEMEMMKMIGKHKNIINLLGACTQDGPLYVIVEYASKGNLREYLRARRPPGMEYSYDINRVPEEQMTFKDLVSCTYQLARGMEYLASQKCIHRDLAARNVLVTENNVMKIADFGLARDINNIDYYKKTTNGRLPVKWMAPEALFDRVYTHQSDVWSFGVLMWEIFTLGGSPYPGIPVEELFKLLKEGHRMDKPANCTNELYMMMRDCWHAVPSQRPTFKQLVEDLDRILTLTTNEEYLDLSQPLEQYSPSYPDTRSSCSSGDDSVFSPDPMPYEPCLPQYPHINGSVKT

SEQ ID NO: 59 - protein, 797 aa, Artificial Sequence
  source: /note="Description of Artificial Sequence: Synthetic polypeptide"
RPSPTLPEQAQPWGAPVEVESFLVHPGDLLQLRCRLRDDVQSINWLRDGVQLAESNRTRITGEEVEVQDSVPADSGLYACVTSSPSGSDTTYFSVNVSDALPSSEDDDDDDDSSSEEKETDNTKPNPVAPYWTSPEKMEKKLHAVPAAKTVKFKCPSSGTPNPTLRWLKNGKEFKPDHRIGGYKVRYATWSIIMDSVVPSDKGNYTCIVENEYGSINHTYQLDVVERSPHRPILQAGLPANKTVALGSNVEFMCKVYSDPQPHIQWLKHIEVNGSKIGPDNLPYVQILKTAGVNTTDKEMEVLHLRNVSFEDAGEYTCLAGNSIGLSHHSAWLTVLEALEERPAVMTSPDYLEIAIYCIGVFLIACMVVTVILCRMKNTTKKPDFSSQPAVHKLTKRIPLRRQVTVSAESSSSMNSNTPLVRITTRLSSTADTPMLAGVSEYELPEDPKWEFPRDKLTLGKPLGEGCFGQVVMAEAVGIDKDKPKEAVTVAVKMLKDDATEKDLSDLVSEMEMMKMIGKHKNIINLLGACTQDGPLYVIVEYASKGNLREYLRARRPPGMEYSYDINRVPEEQMTFKDLVSCTYQLARGMEYLASQKCIHRDLAARNVLVTENNVMKIADFGLARDINNIDYYKKTTNGRLPVKWMAPEALFDRVYTHQSDVWSFGVLMWEIFTLGGSPYPGIPVEELFKLLKEGHRMDKPANCTNELYMMMRDCWHAVPSQRPTFKQLVEDLDRILTLTTNEEYLDLSQPLEQYSPSYPDTRSSCSSGDDSVFSPDPMPYEPCLPQYPHINGSVKT

SEQ ID NO: 60 - protein, 802 aa, Artificial Sequence
  source: /note="Description of Artificial Sequence: Synthetic polypeptide"
RPSFSLVEDTTLEPEEPPTKYQISQPEVYVAAPGESLEVRCLLKDAAVISWTKDGVHLGPNNRTVLIGEYLQIKGATPRDSGLYACTASRTVDSETWYFMVNVTDAISSGDDEDDTDGAEDFVSENSNNKRAPYWTNTEKMEKRLHAVPAANTVKFRCPAGGNPMPTMRWLKNGKEFKQEHRIGGYKVRNQHWSLIMESVVPSDKGNYTCVVENEYGSINHTYHLDVVERSPHRPILQAGLPANASTVVGGDVEFVCKVYSDAQPHIQWIKHVEKNGSKYGPDGLPYLKVLKAAGVNTTDKEIEVLYIRNVTFEDAGEYTCLAGNSIGISFHSAWLTVLPAPGREKEITASPLYLEIIIYCTGAFLISCMVGSVIVYKMKSGTKKSDFHSQMAVHKLAKSIPLRRQVTVSADSSASMNSGVLLVRPSRLSSSGTPMLAGVSEYELPEDPRWELPRDRLVLGKPLGEGCFGQVVLAEAIGLDKDKPNRVTKVAVKMLKSDATEKDLSDLISEMEMMKMIGKHKNIINLLGACTQDGPLYVIVEYASKGNLREYLQARRPPGLEYCYNPSHNPEEQLSSKDLVSCAYQVARGMEYLASKKCIHRDLAARNVLVTEDNVMKIADFGLARDIHHIDYYKKTTNGRLPVKWMAPEALFDRIYTHQSDVWSFGVLLWEIFTLGGSPYPGVPVEELFKLLKEGHRMDKPSNCTNELYMMMRDCWHAVPSQRPTFKQLVEDLDRIVALTSNQEYLDLSMPLDQYSPSFPDTRSSTCSSGEDSVFSHEPLPEEPCLPRHPAQLANGGLKRR

SEQ ID NO: 61 - protein, 797 aa, Artificial Sequence
  source: /note="Description of Artificial Sequence: Synthetic polypeptide"
RPSPTLPEQAQPWGAPVEVESFLVHPGDLLQLRCRLRDDVQSINWLRDGVQLAESNRTRITGEEVEVQDSVPADSGLYACVTSSPSGSDTTYFSVNVSDALPSSEDDDDDDDSSSEEKETDNTKPNPVAPYWTSPEKMEKKLHAVPAAKTVKFKCPSSGTPNPTLRWLKNGKEFKPDHRIGGYKVRYATWSIIMDSVVPSDKGNYTCIVENEYGSINHTYQLDVVERSPHRPILQAGLPANASTVVGGDVEFVCKVYSDAQPHIQWIKHVEKNGSKYGPDGLPYLKVLKAAGVNTTDKEIEVLYIRNVTFEDAGEYTCLAGNSIGISFHSAWLTVLPAPGREKEITASPDYLEIAIYCIGVFLIACMVVTVILCRMKNTTKKPDFSSQPAVHKLTKRIPLRRQVTVSAESSSSMNSNTPLVRITTRLSSTADTPMLAGVSEYELPEDPKWEFPRDKLTLGKPLGEGCFGQVVMAEAVGIDKDKPKEAVTVAVKMLKDDATEKDLSDLVSEMEMMKMIGKHKNIINLLGACTQDGPLYVIVEYASKGNLREYLRARRPPGMEYSYDINRVPEEQMTFKDLVSCTYQLARGMEYLASQKCIHRDLAARNVLVTENNVMKIADFGLARDINNIDYYKKTTNGRLPVKWMAPEALFDRVYTHQSDVWSFGVLMWEIFTLGGSPYPGIPVEELFKLLKEGHRMDKPANCTNELYMMMRDCWHAVPSQRPTFKQLVEDLDRILTLTTNEEYLDLSQPLEQYSPSYPDTRSSCSSGDDSVFSPDPMPYEPCLPQYPHINGSVKT

SEQ ID NO: 62 - protein, 802 aa, Artificial Sequence
  source: /note="Description of Artificial Sequence: Synthetic polypeptide"
RPSFSLVEDTTLEPEEPPTKYQISQPEVYVAAPGESLEVRCLLKDAAVISWTKDGVHLGPNNRTVLIGEYLQIKGATPRDSGLYACTASRTVDSETWYFMVNVTDAISSGDDEDDTDGAEDFVSENSNNKRAPYWTNTEKMEKRLHAVPAANTVKFRCPAGGNPMPTMRWLKNGKEFKQEHRIGGYKVRNQHWSLIMESVVPSDKGNYTCVVENEYGSINHTYHLDVVERSPHRPILQAGLPANKTVALGSNVEFMCKVYSDPQPHIQWLKHIEVNGSKIGPDNLPYVQILKTAGVNTTDKEMEVLHLRNVSFEDAGEYTCLAGNSIGLSHHSAWLTVLEALEERPAVMTSPLYLEIIIYCTGAFLISCMVGSVIVYKMKSGTKKSDFHSQMAVHKLAKSIPLRRQVTVSADSSASMNSGVLLVRPSRLSSSGTPMLAGVSEYELPEDPRWELPRDRLVLGKPLGEGCFGQVVLAEAIGLDKDKPNRVTKVAVKMLKSDATEKDLSDLISEMEMMKMIGKHKNIINLLGACTQDGPLYVIVEYASKGNLREYLQARRPPGLEYCYNPSHNPEEQLSSKDLVSCAYQVARGMEYLASKKCIHRDLAARNVLVTEDNVMKIADFGLARDIHHIDYYKKTTNGRLPVKWMAPEALFDRIYTHQSDVWSFGVLLWEIFTLGGSPYPGVPVEELFKLLKEGHRMDKPSNCTNELYMMMRDCWHAVPSQRPTFKQLVEDLDRIVALTSNQEYLDLSMPLDQYSPSFPDTRSSTCSSGEDSVFSHEPLPEEPCLPRHPAQLANGGLKRR

SEQ ID NO: 63 - DNA, 107 bp, Artificial Sequence
  source: /note="Description of Artificial Sequence: Synthetic primer"
tttccctttatcgattgaattccaccatgggatggtcatgtatcatcctttttctagtagcaactgcaactggagtacattcaactgtggctgcaccatctgtcttc

SEQ ID NO: 64 - DNA, 43 bp, Artificial Sequence
  source: /note="Description of Artificial Sequence: Synthetic primer"
tttccctttaagcttaacactctcccctgttgaagctctttgt

SEQ ID NO: 65 - protein, 107 aa, Homo sapiens [sequence omitted]

SEQ ID NO: 66 - DNA, 321 bp, Homo sapiens
cgaactgtggctgcaccatctgtcttcatcttcccgccatctgatgagcagttgaaatctggaactgcttctgttgtgtgcctgctgaataacttctatccccgtgaggccaaagtacagtggaaggtggataacgccctccaatcgggtaactcccaggagagtgtcacagagcaggacagcaaggacagcacctacagcctcagcagcaccctgacgctgagcaaagcagactacgagaaacacaaagtctacgcctgcgaagtcacccatcagggcctgagctcgcccgtcacaaagagcttcaacaggggagagtgt

SEQ ID NO: 67 - protein, 125 aa, Artificial Sequence
  source: /note="Description of Artificial Sequence: Synthetic polypeptide"
MGWSCIILFLVATATGVHSTVAAPSVFIFPPSDEQLKSGTASVVCLLNNFYPREAKVQWKVDNALQSGNSQESVTEQDSKDSTYSLSSTLTLSKADYEKHKVYACEVTHQGLSSPVTKSFNRGEC

SEQ ID NO: 68 - protein, 20 aa, Artificial Sequence
  source: /note="Description of Artificial Sequence: Synthetic peptide"
GGGGSGGGGSGGGGSGGGGS

SEQ ID NO: 69 - protein, 19 aa, Artificial Sequence
  source: /note="Description of Artificial Sequence: Synthetic peptide"
MGWSCIILFLVATATGAYA

SEQ ID NO: 70 - protein, 5 aa, Artificial Sequence
  source: /note="Description of Artificial Sequence: Synthetic peptide"
GGGGS

SEQ ID NO: 71 - protein, 7 aa, Artificial Sequence
  source: /note="Description of Artificial Sequence: Synthetic peptide"
SGGSGGS

SEQ ID NO: 72 - protein, 9 aa, Artificial Sequence
  source: /note="Description of Artificial Sequence: Synthetic peptide"
GGGGSGGGS

SEQ ID NO: 73 - protein, 10 aa, Artificial Sequence
  source: /note="Description of Artificial Sequence: Synthetic peptide"
GGGGSGGGGS

SEQ ID NO: 74 - protein, 15 aa, Artificial Sequence
  source: /note="Description of Artificial Sequence: Synthetic peptide"
GGGGSGGGGSGGGGS

SEQ ID NO: 75 - protein, 25 aa, Artificial Sequence
  source: /note="Description of Artificial Sequence: Synthetic peptide"
GGGGSGGGGSGGGGSGGGGSGGGGS

SEQ ID NO: 76 - protein, 30 aa, Artificial Sequence
  source: /note="Description of Artificial Sequence: Synthetic polypeptide"
GGGGSGGGGSGGGGSGGGGSGGGGSGGGGS

SEQ ID NO: 77 - protein, 35 aa, Artificial Sequence
  source: /note="Description of Artificial Sequence: Synthetic polypeptide"
GGGGSGGGGSGGGGSGGGGSGGGGSGGGGSGGGGS

SEQ ID NO: 78 - protein, 15 aa, Artificial Sequence
  source: /note="Description of Artificial Sequence: Synthetic peptide"
EPKSCDKTHTCPPCP

SEQ ID NO: 79 - protein, 24 aa, Artificial Sequence
  source: /note="Description of Artificial Sequence: Synthetic peptide"
GGGGSGGGSEPKSCDKTHTCPPCP

SEQ ID NO: 80 - protein, 62 aa, Artificial Sequence
  source: /note="Description of Artificial Sequence: Synthetic polypeptide"
ELKTPLGDTTHTCPRCPEPKSCDTPPPCPRCPEPKSCDTPPPCPRCPEPKSCDTPPPCPRCP

SEQ ID NO: 81 - protein, 6 aa, Artificial Sequence
  source: /note="Description of Artificial Sequence: Synthetic peptide"
GSGSGS

SEQ ID NO: 82 - protein, 3 aa, Artificial Sequence
  source: /note="Description of Artificial Sequence: Synthetic peptide"
AAA

SEQ ID NO: 83 - protein, 6 aa, Artificial Sequence
  source: /note="Description of Artificial Sequence: Synthetic peptide"
ATGAYA

SEQ ID NO: 84 - DNA, 18 bp, Artificial Sequence
  source: /note="Description of Artificial Sequence: Synthetic primer"
atgctctcccctcctcgg

SEQ ID NO: 85 - DNA, 20 bp, Artificial Sequence
  source: /note="Description of Artificial Sequence: Synthetic primer"
aggcccctgtgcaatagatg

SEQ ID NO: 86 - protein, 15 aa, Artificial Sequence
  source: /note="Description of Artificial Sequence: Synthetic peptide"
GGGGSGGGGSGGGGS

SEQ ID NO: 87 - DNA, 23 bp, Artificial Sequence
  source: /note="Description of Artificial Sequence: Synthetic oligonucleotide"
aacttcactgtcttggcagccgg

SEQ ID NO: 88 - DNA, 23 bp, Artificial Sequence
  source: /note="Description of Artificial Sequence: Synthetic oligonucleotide"
gatctccaggtacaggggcgagg